European Patent Application EP 4 458 836 A1, published November 6, 2024. Title: Novel Artificial Nucleic Acids, Production Method Thereof and Use Thereof. Applicant: 株式会社理研ジェネシス. The sequence listing filed with the application follows.

SEQUENCE LISTING (10 sequences)

SEQ ID NO: 1 - DNA, 12 bp, synthetic construct
  modified_base 6: mod_base = OTHER; note = (A)alpha-T, (A)beta-T, (B)beta-T, or (C)Hbeta-T
  source 1..12: mol_type = other DNA; note = antisense strand
gcgttttttgct

SEQ ID NO: 2 - DNA, 12 bp, synthetic construct
  source 1..12: mol_type = other DNA; note = antisense strand
  modified_base 4: mod_base = OTHER; note = (A)alpha-T, (A)beta-T, (B)beta-T, or (C)Hbeta-T
  modified_base 6: mod_base = OTHER; note = (A)alpha-T, (A)beta-T, (B)beta-T, or (C)Hbeta-T
  modified_base 8: mod_base = OTHER; note = (A)alpha-T, (A)beta-T, (B)beta-T, or (C)Hbeta-T
gcgttttttgct

SEQ ID NO: 3 - DNA, 12 bp, synthetic construct
  source 1..12: mol_type = other DNA; note = antisense strand
  modified_base 5..7: mod_base = OTHER; note = (A)alpha-T, (A)beta-T, (B)beta-T, or (C)Hbeta-T
gcgttttttgct

SEQ ID NO: 4 - DNA, 12 bp, synthetic construct
  source 1..12: mol_type = other DNA; note = antisense strand
  modified_base 4..9: mod_base = OTHER; note = (A)alpha-T, (A)beta-T, (B)beta-T, or (C)Hbeta-T
gcgttttttgct

SEQ ID NO: 5 - DNA, 10 bp, synthetic construct
  source 1..10: mol_type = other DNA; note = antisense strand
  modified_base 9: mod_base = OTHER; note = (A)alpha-T, (A)beta-T, (B)beta-T, or (C)Hbeta-T
tttttttttt

SEQ ID NO: 6 - DNA, 12 bp, synthetic construct
  source 1..12: mol_type = other DNA; note = sense strand
  modified_base 7: mod_base = OTHER; note = (C)Hbeta-A
agcaaaaaacgc

SEQ ID NO: 7 - DNA, 12 bp, synthetic construct
  source 1..12: mol_type = other DNA; note = sense strand
agcaaaaaacgc

SEQ ID NO: 8 - RNA, 12 nt, synthetic construct
  source 1..12: mol_type = other RNA; note = sense strand
agcaaaaaacgc

SEQ ID NO: 9 - DNA, 10 bp, synthetic construct
  source 1..10: mol_type = other DNA
tttttttttt

SEQ ID NO: 10 - DNA, 10 bp, synthetic construct
  source 1..10: mol_type = other DNA
  modified_base 9: mod_base = OTHER; note = LNA-T, (A)alpha-T, (A)beta-T, (B)beta-T, or (C)Hbeta-T
tttttttttt